European Patent Application EP 4 292 596 A1, published December 20, 2023. Title: 治疗肿瘤的方法和组合. Applicant: 同润生物医药（上海）有限公司. The sequence listing filed with the application follows.

SEQUENCE LISTING (7 sequences)

SEQ ID NO: 1 - protein, 9 aa, 人工序列（Artificial Sequence）
  HCDR1
GHFSNLAVN

SEQ ID NO: 2 - protein, 17 aa, 人工序列（Artificial Sequence）
  HCDR2
GILWSGGSTFYADSVKG

SEQ ID NO: 3 - protein, 3 aa, 人工序列（Artificial Sequence）
  HCDR3
GTN

SEQ ID NO: 4 - protein, 111 aa, 人工序列（Artificial Sequence）
  VHH
EVQLVESGGGLVQPGGSLRLSCAASGHFSNLAVNWFRQAPGKERELVAGILWSGGSTFYADSVKGRFTISRGNAENMLYLQMNSLRAEDTAVYYCNTGTNWGQGTLVTVSS

SEQ ID NO: 5 - protein, 20 aa, 人工序列（Artificial Sequence）
  肽连接子
GGGGSGGGGSGGGGSGGGGS

SEQ ID NO: 6 - protein, 136 aa, 人工序列（Artificial Sequence）
  TGFβRII 胞外结构域
IPPHVQKSVNNDMIVTDNNGAVKFPQLCKFCDVRFSTCDNQKSCMSNCSITSICEKPQEVCVAVWRKNDENITLETVCHDPKLPYHDFILEDAASPKCIMKEKKKPGETFFMCSCSSDECNDNIIFSEEYNTSNPD

SEQ ID NO: 7 - protein, 497 aa, 人工序列（Artificial Sequence）
  多肽
EVQLVESGGGLVQPGGSLRLSCAASGHFSNLAVNWFRQAPGKERELVAGILWSGGSTFYADSVKGRFTISRGNAENMLYLQMNSLRAEDTAVYYCNTGTNWGQGTLVTVSSEPKSCDKTHTCPPCPAPELLGGPSVFLFPPKPKDTLMISRTPEVTCVVVDVSHEDPEVKFNWYVDGVEVHNAKTKPREEQYNSTYRVVSVLTVLHQDWLNGKEYKCKVSNKALPAPIEKTISKAKGQPREPQVYTLPPSREEMTKNQVSLTCLVKGFYPSDIAVEWESNGQPENNYKTTPPVLDSDGSFFLYSKLTVDKSRWQQGNVFSCSVMHEALHNHYTQKSLSLSPGGGGSGGGGSGGGGSGGGGSIPPHVQKSVNNDMIVTDNNGAVKFPQLCKFCDVRFSTCDNQKSCMSNCSITSICEKPQEVCVAVWRKNDENITLETVCHDPKLPYHDFILEDAASPKCIMKEKKKPGETFFMCSCSSDECNDNIIFSEEYNTSNPD